European Patent Application EP 4 527 401 A1, published March 26, 2025. Title: Method for producing a hot-water extract from the aerial part of Araliaceae, composition for promoting expression of uroguanylin or guanylin, composition for promoting intestinal peristalsis, composition for suppressing intestinal inflammation, and composition for improving intestinal barrier function. Applicant: 株式会社アミノアップ. The sequence listing filed with the application follows.

SEQUENCE LISTING (20 sequences)

SEQ ID NO: 1 - DNA, 20 bp, synthetic construct
  source 1..20: mol_type = other DNA
  misc_feature 1..20: note = uroguanylin gene primer 1
gctgcagagcacacagtcag

SEQ ID NO: 2 - DNA, 20 bp, synthetic construct
  source 1..20: mol_type = other DNA
  misc_feature 1..20: note = uroguanylin gene primer 2
tgtgcctccaggtcactcag

SEQ ID NO: 3 - DNA, 20 bp, synthetic construct
  source 1..20: mol_type = other DNA
  misc_feature 1..20: note = guanylin gene primer 1
gatactccactcccagcagc

SEQ ID NO: 4 - DNA, 20 bp, synthetic construct
  source 1..20: mol_type = other DNA
  misc_feature 1..20: note = guanylin gene primer 2
ttgaagtggcagggaaggac

SEQ ID NO: 5 - DNA, 21 bp, synthetic construct
  source 1..21: mol_type = other DNA
  misc_feature 1..21: note = GAPDH gene primer 1
gaaggtcggagtcaacggatt

SEQ ID NO: 6 - DNA, 20 bp, synthetic construct
  source 1..20: mol_type = other DNA
  misc_feature 1..20: note = GAPDH gene primer 2
cgctcctggaagatggtgat

SEQ ID NO: 7 - DNA, 20 bp, synthetic construct
  source 1..20: mol_type = other DNA
  misc_feature 1..20: note = uroguanylin gene primer 1
aggagatgtccaatccccag

SEQ ID NO: 8 - DNA, 21 bp, synthetic construct
  source 1..21: mol_type = other DNA
  misc_feature 1..21: note = uroguanylin gene primer 2
acagttcacattcgtcggtgg

SEQ ID NO: 9 - DNA, 20 bp, synthetic construct
  source 1..20: mol_type = other DNA
  misc_feature 1..20: note = guanylin gene primer 1
gatcctgcagaggctagagg

SEQ ID NO: 10 - DNA, 20 bp, synthetic construct
  source 1..20: mol_type = other DNA
  misc_feature 1..20: note = guanylin gene primer 2
aaggcaagcgatgtcactct

SEQ ID NO: 11 - DNA, 20 bp, synthetic construct
  source 1..20: mol_type = other DNA
  misc_feature 1..20: note = GAPDH gene primer 1
acccagaagactgtggatgg

SEQ ID NO: 12 - DNA, 20 bp, synthetic construct
  source 1..20: mol_type = other DNA
  misc_feature 1..20: note = GAPDH gene primer 2
tcagctctgggatgaccttg

SEQ ID NO: 13 - DNA, 22 bp, synthetic construct
  source 1..22: mol_type = other DNA
  misc_feature 1..22: note = calprotectin gene primer 1
tgagtgtcctcagtttgtgcag

SEQ ID NO: 14 - DNA, 22 bp, synthetic construct
  source 1..22: mol_type = other DNA
  misc_feature 1..22: note = calprotectin gene primer 2
tgtgagatgccacacccacttt

SEQ ID NO: 15 - DNA, 19 bp, synthetic construct
  source 1..19: mol_type = other DNA
  misc_feature 1..19: note = claudin 4 gene primer 1
cgctactcttgccattacg

SEQ ID NO: 16 - DNA, 20 bp, synthetic construct
  source 1..20: mol_type = other DNA
  misc_feature 1..20: note = claudin 4 gene primer 2
actcagcacaccatgacttg

SEQ ID NO: 17 - DNA, 20 bp, synthetic construct
  source 1..20: mol_type = other DNA
  misc_feature 1..20: note = JAM-A gene primer 1
accctccctcctttccttac

SEQ ID NO: 18 - DNA, 20 bp, synthetic construct
  source 1..20: mol_type = other DNA
  misc_feature 1..20: note = JAM-A gene primer 2
ctaggactcttgcccaatcc

SEQ ID NO: 19 - DNA, 20 bp, synthetic construct
  source 1..20: mol_type = other DNA
  misc_feature 1..20: note = occludin gene primer 1
ttgacagtccaatggcctac

SEQ ID NO: 20 - DNA, 21 bp, synthetic construct
  source 1..21: mol_type = other DNA
  misc_feature 1..21: note = occludin gene primer 2
catccacactcaaggtcagag